European Patent Application EP 4 190 913 A1, published June 7, 2023. Title: FUNCTIONALIZED METAL NANOPARTICLES AND USES THEREOF FOR DETECTING SARS CoV 2 GENETIC MATERIAL. Applicant: FUNDACIÓN IMDEA NANOCIENCIA. The sequence listing filed with the application follows.

SEQUENCE LISTING (32 sequences)

SEQ ID NO: 1 - DNA, 26 bp, Artificial Sequence
  E gene target region
acactagccatccttactgcgcttcg

SEQ ID NO: 2 - RNA, 26 nt, Artificial Sequence
  E gene target region RNA
acacuagccauccuuacugcgcuucg

SEQ ID NO: 3 - DNA, 24 bp, Artificial Sequence
  ORBab1 target region DNA
caggtggaacctcatcaggagatg

SEQ ID NO: 4 - RNA, 24 nt, Artificial Sequence
  ORF1ab target region RNA
cagguggaaccucaucaggagaug

SEQ ID NO: 5 - DNA, 27 bp, Artificial Sequence
  S gene target region DNA
ctaattctcctcggcgggcacgtagtg

SEQ ID NO: 6 - RNA, 27 nt, Artificial Sequence
  S gene target region RNA
cuaauucuccucggcgggcacguagug

SEQ ID NO: 7 - DNA, 15 bp, Artificial Sequence
  S gene D residue target region DNA
tatcaggatgttaac

SEQ ID NO: 8 - RNA, 15 nt, Artificial Sequence
  S gene D residue target region RNA
uaucaggauguuaac

SEQ ID NO: 9 - DNA, 15 bp, Artificial Sequence
  S gene D residue target region DNA
tatcagggtgttaac

SEQ ID NO: 10 - RNA, 15 nt, Artificial Sequence
  S gene D residue target region RNA
uaucaggguguuaac

SEQ ID NO: 11 - DNA, 25 bp, Artificial Sequence
  S gene D residue target region DNA
ttctttatcagggtgttaactgcac

SEQ ID NO: 12 - RNA, 25 nt, Artificial Sequence
  S gene D residue target region RNA
uucuuuaucaggguguuaacugcac

SEQ ID NO: 13 - DNA, 39 bp, Artificial Sequence
  Nanoparticle attached oligonucleotide
tttttcggccgaagcgcagtaaggatggctagtgtgccg

SEQ ID NO: 14 - DNA, 41 bp, Artificial Sequence
  Nanoparticle attached oligonucleotide
tttttcggcccgaagcgcagtaaggatggctagtgtggccg

SEQ ID NO: 15 - DNA, 43 bp, Artificial Sequence
  Nanoparticle attached oligonucleotide
tttttgcggcccgaagcgcagtaaggatggctagtgtggccgc

SEQ ID NO: 16 - DNA, 38 bp, Artificial Sequence
  Nanoparticle attached oligonucleotide
tttttcggcgcatctcctgatgaggttccacctggccg

SEQ ID NO: 17 - DNA, 40 bp, Artificial Sequence
  Nanoparticle attached oligonucleotide
tttttcggccgcatctcctgatgaggttccacctgggccg

SEQ ID NO: 18 - DNA, 42 bp, Artificial Sequence
  Nanoaparticle attached oligonucleotide
tttttgcggccgcatctcctgatgaggttccacctgggccgc

SEQ ID NO: 19 - DNA, 42 bp, Artificial Sequence
  Nanoparticle attached oligonucleotide
tttttcggcccactacgtgcccgccgaggagaattagggccg

SEQ ID NO: 20 - DNA, 30 bp, Artificial Sequence
  Nanoapraticle attached oligonucleotide
tttttcagtcgttaacatcctgatagactg

SEQ ID NO: 21 - DNA, 30 bp, Artificial Sequence
  Nanoparticle attached oligonucleotide
tttttcagtcgttaacaccctgatagactg

SEQ ID NO: 22 - DNA, 40 bp, Artificial Sequence
  Nanoparticle attached oligonucleotide
tttttcagtcgtgcagttaacaccctgataaagaagactg

SEQ ID NO: 23 - DNA, 23 bp, Artificial Sequence
  Influenza virus A target region
cttctaaccgaggtcgaaacgta

SEQ ID NO: 24 - DNA, 22 bp, Artificial Sequence
  Ingluenza virus B target region
tgcctacctgctttcactaaca

SEQ ID NO: 25 - DNA, 18 bp, Artificial Sequence
  Mycoplasma pneumoniae target region
gaattccatgacatggta

SEQ ID NO: 26 - DNA, 24 bp, Artificial Sequence
  Legionalla pneumoniae target region
gacaaggataagttgtcttatagc

SEQ ID NO: 27 - DNA, 22 bp, Artificial Sequence
  R fragment forward primer
  misc_feature (1)..(6): phosphorothioate bond
gtgtggcggttcactatatgtt

SEQ ID NO: 28 - DNA, 24 bp, Artificial Sequence
  R fragment reverse primer
gcactattagcataagcagttgtg

SEQ ID NO: 29 - DNA, 22 bp, Artificial Sequence
  E fragment forward primer
  misc_feature (1)..(6): phosphorothioate bond
gctttcgtggtattcttgctag

SEQ ID NO: 30 - DNA, 22 bp, Artificial Sequence
  E fragment reverse primer
atattgcagcagtacgcacaca

SEQ ID NO: 31 - DNA, 22 bp, Artificial Sequence
  S fragment forward primer
  misc_feature (1)..(6): phosphorothioate bond
caaatacttctaaccaggttgc

SEQ ID NO: 32 - DNA, 22 bp, Artificial Sequence
  S fragment reverse primer
catgaatagcaacagggacttc